European Patent Application EP 4 474 480 A2, published December 11, 2024. Title: COMBINED TELOMERASE INHIBITOR AND GEMCITABINE FOR THE TREAMENT OF CANCER. Applicant: Geron Corporation. Application EP. The sequence listing filed with the application follows.

SEQUENCE LISTING (27 sequences)

SEQ ID NO: 1 - RNA, 554 nt, Homo sapiens
  source 1..554: mol_type = other RNA
gggttgcggagggtgggcctgggaggggtggtggccattttttgtctaaccctaactgagaagggcgtaggcgccgtgcttttgctccccgcgcgctgtttttctcgctgactttcagcgggcggaaaagcctcggcctgccgccttccaccgttcattctagagcaaacaaaaaatgtcagctgctggcccgttcgcctcccggggacctgcggcgggtcgcctgcccagcccccgaaccccgcctggagccgcggtcggcccggggcttctccggaggcacccactgccaccgcgaagagttgggctctgtcagccgcgggtctctcgggggcgagggcgaggttcaccgtttcaggccgcaggaagaggaacggagcgagtcccgccgcggcgcgattccctgagctgtgggacgtgcacccaggactcggctcacacatgcagttcgctttcctgttggtggggggaacgccgatcgtgcgcatccgtcacccctcgccggcagtgggggcttgtgaacccccaaacctgactgactgggccagtgtgct

SEQ ID NO: 2 - DNA, 20 bp, synthetic construct
  misc_feature 1..20: note = Oligonucleotide
  source 1..20: mol_type = other DNA
acattttttgtttgctctag

SEQ ID NO: 3 - DNA, 30 bp, synthetic construct
  misc_feature 1..30: note = Oligonucleotide
  source 1..30: mol_type = other DNA
gctctagaatgaacggtggaaggcggcagg

SEQ ID NO: 4 - DNA, 14 bp, synthetic construct
  misc_feature 1..14: note = Oligonucleotide
  source 1..14: mol_type = other DNA
gtggaggcggcagg

SEQ ID NO: 5 - DNA, 13 bp, synthetic construct
  misc_feature 1..13: note = Oligonucleotide
  source 1..13: mol_type = other DNA
ggaaggcggcagg

SEQ ID NO: 6 - DNA, 13 bp, synthetic construct
  misc_feature 1..13: note = Oligonucleotide
  source 1..13: mol_type = other DNA
gtggaaggcggca

SEQ ID NO: 7 - DNA, 11 bp, synthetic construct
  misc_feature 1..11: note = Oligonucleotide
  source 1..11: mol_type = other DNA
gtggaaggcgg

SEQ ID NO: 8 - DNA, 13 bp, synthetic construct
  misc_feature 1..13: note = Oligonucleotide
  source 1..13: mol_type = other DNA
cggtggaaggcgg

SEQ ID NO: 9 - DNA, 13 bp, synthetic construct
  misc_feature 1..13: note = Oligonucleotide
  source 1..13: mol_type = other DNA
acggtggaaggcg

SEQ ID NO: 10 - DNA, 16 bp, synthetic construct
  misc_feature 1..16: note = Oligonucleotide
  source 1..16: mol_type = other DNA
aacggtggaaggcggc

SEQ ID NO: 11 - DNA, 18 bp, synthetic construct
  misc_feature 1..18: note = Oligonucleotide
  source 1..18: mol_type = other DNA
atgaacggtggaaggcgg

SEQ ID NO: 12 - DNA, 13 bp, synthetic construct
  misc_feature 1..13: note = Oligonucleotide
  source 1..13: mol_type = other DNA
tagggttagacaa

SEQ ID NO: 13 - DNA, 13 bp, synthetic construct
  misc_feature 1..13: note = Oligonucleotide
  source 1..13: mol_type = other DNA
cagttagggttag

SEQ ID NO: 14 - DNA, 12 bp, synthetic construct
  misc_feature 1..12: note = Oligonucleotide
  source 1..12: mol_type = other DNA
tagggttagaca

SEQ ID NO: 15 - DNA, 11 bp, synthetic construct
  misc_feature 1..11: note = Oligonucleotide
  source 1..11: mol_type = other DNA
tagggttagac

SEQ ID NO: 16 - DNA, 11 bp, synthetic construct
  misc_feature 1..11: note = Oligonucleotide
  source 1..11: mol_type = other DNA
gttagggttag

SEQ ID NO: 17 - DNA, 13 bp, synthetic construct
  misc_feature 1..13: note = Oligonucleotide
  source 1..13: mol_type = other DNA
gttagggttagac

SEQ ID NO: 18 - DNA, 15 bp, synthetic construct
  misc_feature 1..15: note = Oligonucleotide
  source 1..15: mol_type = other DNA
gttagggttagacaa

SEQ ID NO: 19-20 - skipped (2 entries)

SEQ ID NO: 21 - DNA, 12 bp, synthetic construct
  misc_feature 1..12: note = Oligonucleotide
  source 1..12: mol_type = other DNA
cccttctcagtt

SEQ ID NO: 22 - DNA, 12 bp, synthetic construct
  misc_feature 1..12: note = Oligonucleotide
  source 1..12: mol_type = other DNA
cgcccttctcag

SEQ ID NO: 23 - DNA, 13 bp, synthetic construct
  misc_feature 1..13: note = Oligonucleotide
  source 1..13: mol_type = other DNA
taggtgtaagcaa

SEQ ID NO: 24 - DNA, 13 bp, synthetic construct
  misc_feature 1..13: note = Oligonucleotide
  source 1..13: mol_type = other DNA
ttgtctaacccta

SEQ ID NO: 25 - DNA, 11 bp, synthetic construct
  misc_feature 1..11: note = Oligonucleotide
  source 1..11: mol_type = other DNA
gttgagtgtag

SEQ ID NO: 26 - skipped

SEQ ID NO: 27 - DNA, 10 bp, synthetic construct
  misc_feature 1..10: note = Oligonucleotide
  source 1..10: mol_type = other DNA
tttttttttt